European Patent Application EP 4 238 989 A1, published September 6, 2023. Title: ANTI-IL5 NANOANTIBODY AND USE THEREOF. Applicant: SHANGHAI NOVAMAB BIOPHARMACEUTICALS CO., LTD. The sequence listing filed with the application follows.

SEQUENCE LISTING (63 sequences)

SEQ ID NO: 1 - protein, 11 aa, Camelus bactrianus
GYPYSGDYCMG

SEQ ID NO: 2 - protein, 8 aa, Camelus bactrianus
FYTGGGST

SEQ ID NO: 3 - protein, 24 aa, Camelus bactrianus
AADPWSVYGGSCGVKDPNPKAFNY

SEQ ID NO: 4 - protein, 25 aa, Camelus bactrianus
QVQLQESGGGSAQAGGSLKLSCVVS

SEQ ID NO: 5 - protein, 15 aa, Camelus bactrianus
WFRQAPGKEREGVAA

SEQ ID NO: 6 - protein, 38 aa, Camelus bactrianus
YYADSVKGRFTTSQDNATSTFHLQMNSLKPEDTATYYC

SEQ ID NO: 7 - protein, 11 aa, Camelus bactrianus
WGQGTQVTVSS

SEQ ID NO: 8 - protein, 132 aa, Camelus bactrianus
QVQLQESGGGSAQAGGSLKLSCVVSGYPYSGDYCMGWFRQAPGKEREGVAAFYTGGGSTYYADSVKGRFTTSQDNATSTFHLQMNSLKPEDTATYYCAADPWSVYGGSCGVKDPNPKAFNYWGQGTQVTVSS

SEQ ID NO: 9 - DNA, 396 bp, Camelus bactrianus
caggtgcagctgcaggagtctgggggaggctcggcgcaggctggagggtctctgaaactctcctgtgtagtctctggatacccctacagtggcgattactgcatgggctggttccgccaggctccagggaaggagcgcgagggggtcgcagcgttttatactggtggtggtagcacatactatgccgactccgtgaagggccgattcaccacctcccaagacaacgccacgagcacgtttcatctgcaaatgaacagcctgaaacctgaggacactgccacgtactactgcgcggcagacccgtggagtgtgtacggtggtagctgtggggtaaaagatcccaatccgaaggcctttaattactggggccaggggacccaggtcaccgtctcctca

SEQ ID NO: 10 - protein, 10 aa, Camelus bactrianus
EYTYSRYCMG

SEQ ID NO: 11 - protein, 7 aa, Camelus bactrianus
IDSDGST

SEQ ID NO: 12 - protein, 22 aa, Camelus bactrianus
AARYFYIATTGLRPCGEYEYNY

SEQ ID NO: 13 - protein, 25 aa, Camelus bactrianus
QVQLQESGGGSVQAGGSLRLSCAAS

SEQ ID NO: 14 - protein, 15 aa, Camelus bactrianus
WFRQVPGKEREGVAT

SEQ ID NO: 15 - protein, 38 aa, Camelus bactrianus
SYADSVKGRFTISKDNAKNTLYLQMNSLKPEDTAMYYC

SEQ ID NO: 16 - protein, 11 aa, Camelus bactrianus
WGQGTQVTVSS

SEQ ID NO: 17 - protein, 128 aa, Camelus bactrianus
QVQLQESGGGSVQAGGSLRLSCAASEYTYSRYCMGWFRQVPGKEREGVATIDSDGSTSYADSVKGRFTISKDNAKNTLYLQMNSLKPEDTAMYYCAARYFYIATTGLRPCGEYEYNYWGQGTQVTVSS

SEQ ID NO: 18 - DNA, 384 bp, Camelus bactrianus
caggtgcagctgcaggagtctggaggaggctcggtgcaggctggagggtctctgagactctcctgtgcagcctctgaatacacctacagtagatactgcatgggctggttccgtcaggttccagggaaggagcgcgagggggtcgcaactattgatagtgatggtagcacaagctacgcagactccgtgaagggccgattcaccatctccaaagacaacgccaagaacactctgtatctgcaaatgaacagcctgaaacctgaggacactgccatgtactactgtgcggcccgatacttttatatagcgactacgggcctgagaccctgcggggaatatgagtataactactggggccaggggacccaggtcaccgtctcctca

SEQ ID NO: 19 - protein, 9 aa, Camelus bactrianus
GYTVSSNMG

SEQ ID NO: 20 - protein, 7 aa, Camelus bactrianus
IYPDGAT

SEQ ID NO: 21 - protein, 17 aa, Camelus bactrianus
AADLAFNGLGTLALHGY

SEQ ID NO: 22 - protein, 25 aa, Camelus bactrianus
QVQLQESGGGSVQAGGSLRLSCAAS

SEQ ID NO: 23 - protein, 15 aa, Camelus bactrianus
WFRQAPGKEREGVAA

SEQ ID NO: 24 - protein, 38 aa, Camelus bactrianus
YYADSVKGRFTISQDNAENTVYLQMNSLKPEDTAMYYC

SEQ ID NO: 25 - protein, 11 aa, Camelus bactrianus
WGQGTQVTVSS

SEQ ID NO: 26 - protein, 122 aa, Camelus bactrianus
QVQLQESGGGSVQAGGSLRLSCAASGYTVSSNMGWFRQAPGKEREGVAAIYPDGATYYADSVKGRFTISQDNAENTVYLQMNSLKPEDTAMYYCAADLAFNGLGTLALHGYWGQGTQVTVSS

SEQ ID NO: 27 - DNA, 366 bp, Camelus bactrianus
caggtgcagctgcaggagtctgggggaggctcggtgcaggctggagggtctctgagactctcctgtgcagcctctggatacaccgtcagtagcaacatgggctggttccgccaggctccagggaaggagcgcgagggggtcgcagctatttatcctgatggtgccacatactatgccgactccgtgaagggccgattcaccatctcccaagacaacgccgagaacacggtgtatctgcaaatgaacagcctgaaacctgaggacactgccatgtactactgtgcggcagacctcgcctttaatgggttgggtactctcgcattacatggttactggggccaggggacccaggtcaccgtctcctca

SEQ ID NO: 28 - protein, 10 aa, Camelus bactrianus
GFTFSNYYMS

SEQ ID NO: 29 - protein, 8 aa, Camelus bactrianus
ISSDGSNT

SEQ ID NO: 30 - protein, 12 aa, Camelus bactrianus
ATDLYDDSWYDH

SEQ ID NO: 31 - protein, 25 aa, Camelus bactrianus
QVQLQESGGGLVQPGGSLRLSCAAS

SEQ ID NO: 32 - protein, 15 aa, Camelus bactrianus
WVRQAPGKGLEWVSS

SEQ ID NO: 33 - protein, 38 aa, Camelus bactrianus
YYEDSVKGRFTISRDNANNTLYLQMNSLKSEDTALYHC

SEQ ID NO: 34 - protein, 11 aa, Camelus bactrianus
WGQGTQVTVSS

SEQ ID NO: 35 - protein, 119 aa, Camelus bactrianus
QVQLQESGGGLVQPGGSLRLSCAASGFTFSNYYMSWVRQAPGKGLEWVSSISSDGSNTYYEDSVKGRFTISRDNANNTLYLQMNSLKSEDTALYHCATDLYDDSWYDHWGQGTQVTVSS

SEQ ID NO: 36 - DNA, 357 bp, Camelus bactrianus
caggtgcagctgcaggagtctggaggaggcttggtgcagcctggggggtctctgagactctcctgtgcagcctctggattcaccttcagtaactactacatgagctgggtccgccaggctccagggaaggggctggagtgggtgtccagtattagtagtgatggtagtaacacatactatgaagactccgtgaagggccgattcaccatctccagagacaacgccaataacaccttgtatctgcaaatgaacagcctgaaatctgaggacacggccctgtatcactgtgccactgatctctacgatgatagctggtacgatcactggggccaggggacccaggtcaccgtctcctca

SEQ ID NO: 37 - protein, 25 aa, Artificial Sequence
  HuNb21 FR1
EVQLQESGGGLVQPGGSLRLSCAAS

SEQ ID NO: 38 - protein, 15 aa, Artificial Sequence
  HuNb21 FR2
WFRQAPGKEREGVAA

SEQ ID NO: 39 - protein, 38 aa, Artificial Sequence
  HuNb21 FR3
YYADSVKGRFTISRDNSKNTLYLQMNSLRAEDTAVYYC

SEQ ID NO: 40 - protein, 11 aa, Artificial Sequence
  HuNb21 FR4
WGQGTLVTVSS

SEQ ID NO: 41 - protein, 132 aa, Artificial Sequence
  HuNb21 amino acid sequence
EVQLQESGGGLVQPGGSLRLSCAASGYPYSGDYCMGWFRQAPGKEREGVAAFYTGGGSTYYADSVKGRFTISRDNSKNTLYLQMNSLRAEDTAVYYCAADPWSVYGGSCGVKDPNPKAFNYWGQGTLVTVSS

SEQ ID NO: 42 - DNA, 396 bp, Artificial Sequence
  HuNb21 nucleotide sequence
gaggtgcagctgcaggagagcggcggcggcctggtgcagcccggcggcagcctgaggctgagctgcgccgccagcggctacccctacagcggcgactactgcatgggctggttcaggcaggcccccggcaaggagagggagggcgtggccgccttctacaccggcggcggcagcacctactacgccgacagcgtgaagggcaggttcaccatcagcagggacaacagcaagaacaccctgtacctgcagatgaacagcctgagggccgaggacaccgccgtgtactactgcgccgccgacccctggagcgtgtacggcggcagctgcggcgtgaaggaccccaaccccaaggccttcaactactggggccagggcaccctggtgaccgtgagcagc

SEQ ID NO: 43 - protein, 25 aa, Artificial Sequence
  HuNb66 FR1
EVQLQESGGGLVQPGGSLRLSCAAS

SEQ ID NO: 44 - protein, 15 aa, Artificial Sequence
  HuNb66 FR2
WFRQAPGKEREGVAA

SEQ ID NO: 45 - protein, 38 aa, Artificial Sequence
  HuNb66 FR3
YYADSVKGRFTISRDNSENTLYLQMNSLRAEDTAMYYC

SEQ ID NO: 46 - protein, 11 aa, Artificial Sequence
  HuNb66 FR4
WGQGTLVTVSS

SEQ ID NO: 47 - protein, 122 aa, Artificial Sequence
  HuNb66 amino acid sequence
EVQLQESGGGLVQPGGSLRLSCAASGYTVSSNMGWFRQAPGKEREGVAAIYPDGATYYADSVKGRFTISRDNSENTLYLQMNSLRAEDTAMYYCAADLAFNGLGTLALHGYWGQGTLVTVSS

SEQ ID NO: 48 - DNA, 366 bp, Artificial Sequence
  HuNb66 nucleotide sequence
gaggtgcagctgcaggagagcggcggcggcctggtgcagcccggcggcagcctgaggctgagctgcgccgccagcggctacaccgtgagcagcaacatgggctggttcaggcaggcccccggcaaggagagggagggcgtggccgccatctaccccgacggcgccacctactacgccgacagcgtgaagggcaggttcaccatcagcagggacaacagcgagaacaccctgtacctgcagatgaacagcctgagggccgaggacaccgccatgtactactgcgccgccgacctggccttcaacggcctgggcaccctggccctgcacggctactggggccagggcaccctggtgaccgtgagcagc

SEQ ID NO: 49 - protein, 364 aa, Artificial Sequence
  HuNb21-Fc amino acid sequence
EVQLQESGGGLVQPGGSLRLSCAASGYPYSGDYCMGWFRQAPGKEREGVAAFYTGGGSTYYADSVKGRFTISRDNSKNTLYLQMNSLRAEDTAVYYCAADPWSVYGGSCGVKDPNPKAFNYWGQGTLVTVSSEPKSCDKTHTCPPCPAPELLGGPSVFLFPPKPKDTLMISRTPEVTCVVVDVSHEDPEVKFNWYVDGVEVHNAKTKPREEQYNSTYRVVSVLTVLHQDWLNGKEYKCKVSNKALPAPIEKTISKAKGQPREPQVYTLPPSREEMTKNQVSLTCLVKGFYPSDIAVEWESNGQPENNYKTTPPVLDSDGSFFLYSKLTVDKSRWQQGNVFSCSVMHEALHNHYTQKSLSLSPGK

SEQ ID NO: 50 - DNA, 1092 bp, Artificial Sequence
  HuNb21-Fc nucleotide sequence
gaggtgcagctgcaggagagcggcggcggcctggtgcagcccggcggcagcctgaggctgagctgcgccgccagcggctacccctacagcggcgactactgcatgggctggttcaggcaggcccccggcaaggagagggagggcgtggccgccttctacaccggcggcggcagcacctactacgccgacagcgtgaagggcaggttcaccatcagcagggacaacagcaagaacaccctgtacctgcagatgaacagcctgagggccgaggacaccgccgtgtactactgcgccgccgacccctggagcgtgtacggcggcagctgcggcgtgaaggaccccaaccccaaggccttcaactactggggccagggcaccctggtgaccgtgagcagcgagcccaagagctgcgacaagacccacacctgccccccctgccccgcccccgagctgctgggcggccccagcgtgttcctgttcccccccaagcccaaggacaccctgatgatcagcaggacccccgaggtgacctgcgtggtggtggacgtgagccacgaggaccccgaggtgaagttcaactggtacgtggacggcgtggaggtgcacaacgccaagaccaagcccagggaggagcagtacaacagcacctacagggtggtgagcgtgctgaccgtgctgcaccaggactggctgaacggcaaggagtacaagtgcaaggtgagcaacaaggccctgcccgcccccatcgagaagaccatcagcaaggccaagggccagcccagggagccccaggtgtacaccctgccccccagcagggaggagatgaccaagaaccaggtgagcctgacctgcctggtgaagggcttctaccccagcgacatcgccgtggagtgggagagcaacggccagcccgagaacaactacaagaccaccccccccgtgctggacagcgacggcagcttcttcctgtacagcaagctgaccgtggacaagagcaggtggcagcagggcaacgtgttcagctgcagcgtgatgcacgaggccctgcacaaccactacacccagaagagcctgagcctgagccccggcaag

SEQ ID NO: 51 - protein, 354 aa, Artificial Sequence
  HuNb66-Fc amino acid sequence
EVQLQESGGGLVQPGGSLRLSCAASGYTVSSNMGWFRQAPGKEREGVAAIYPDGATYYADSVKGRFTISRDNSENTLYLQMNSLRAEDTAMYYCAADLAFNGLGTLALHGYWGQGTLVTVSSEPKSCDKTHTCPPCPAPELLGGPSVFLFPPKPKDTLMISRTPEVTCVVVDVSHEDPEVKFNWYVDGVEVHNAKTKPREEQYNSTYRVVSVLTVLHQDWLNGKEYKCKVSNKALPAPIEKTISKAKGQPREPQVYTLPPSREEMTKNQVSLTCLVKGFYPSDIAVEWESNGQPENNYKTTPPVLDSDGSFFLYSKLTVDKSRWQQGNVFSCSVMHEALHNHYTQKSLSLSPGK

SEQ ID NO: 52 - DNA, 1062 bp, Artificial Sequence
  HuNb66-Fc nucleotide sequence
gaggtgcagctgcaggagagcggcggcggcctggtgcagcccggcggcagcctgaggctgagctgcgccgccagcggctacaccgtgagcagcaacatgggctggttcaggcaggcccccggcaaggagagggagggcgtggccgccatctaccccgacggcgccacctactacgccgacagcgtgaagggcaggttcaccatcagcagggacaacagcgagaacaccctgtacctgcagatgaacagcctgagggccgaggacaccgccatgtactactgcgccgccgacctggccttcaacggcctgggcaccctggccctgcacggctactggggccagggcaccctggtgaccgtgagcagcgagcccaagagctgcgacaagacccacacctgccccccctgccccgcccccgagctgctgggcggccccagcgtgttcctgttcccccccaagcccaaggacaccctgatgatcagcaggacccccgaggtgacctgcgtggtggtggacgtgagccacgaggaccccgaggtgaagttcaactggtacgtggacggcgtggaggtgcacaacgccaagaccaagcccagggaggagcagtacaacagcacctacagggtggtgagcgtgctgaccgtgctgcaccaggactggctgaacggcaaggagtacaagtgcaaggtgagcaacaaggccctgcccgcccccatcgagaagaccatcagcaaggccaagggccagcccagggagccccaggtgtacaccctgccccccagcagggaggagatgaccaagaaccaggtgagcctgacctgcctggtgaagggcttctaccccagcgacatcgccgtggagtgggagagcaacggccagcccgagaacaactacaagaccaccccccccgtgctggacagcgacggcagcttcttcctgtacagcaagctgaccgtggacaagagcaggtggcagcagggcaacgtgttcagctgcagcgtgatgcacgaggccctgcacaaccactacacccagaagagcctgagcctgagccccggcaag

SEQ ID NO: 53 - protein, 516 aa, Artificial Sequence
  HuNb21-HuNb21-Fc amino acid sequence
EVQLQESGGGLVQPGGSLRLSCAASGYPYSGDYCMGWFRQAPGKEREGVAAFYTGGGSTYYADSVKGRFTISRDNSKNTLYLQMNSLRAEDTAVYYCAADPWSVYGGSCGVKDPNPKAFNYWGQGTLVTVSSGGGGSGGGGSGGGGSGGGGSEVQLQESGGGLVQPGGSLRLSCAASGYPYSGDYCMGWFRQAPGKEREGVAAFYTGGGSTYYADSVKGRFTISRDNSKNTLYLQMNSLRAEDTAVYYCAADPWSVYGGSCGVKDPNPKAFNYWGQGTLVTVSSEPKSCDKTHTCPPCPAPELLGGPSVFLFPPKPKDTLMISRTPEVTCVVVDVSHEDPEVKFNWYVDGVEVHNAKTKPREEQYNSTYRVVSVLTVLHQDWLNGKEYKCKVSNKALPAPIEKTISKAKGQPREPQVYTLPPSREEMTKNQVSLTCLVKGFYPSDIAVEWESNGQPENNYKTTPPVLDSDGSFFLYSKLTVDKSRWQQGNVFSCSVMHEALHNHYTQKSLSLSPGK

SEQ ID NO: 54 - DNA, 1548 bp, Artificial Sequence
  HuNb21-HuNb21-Fc nucleotide sequence
gaggtgcagctgcaggagagcggcggcggcctggtgcagcccggcggcagcctgaggctgagctgcgccgccagcggctacccctacagcggcgactactgcatgggctggttcaggcaggcccccggcaaggagagggagggcgtggccgccttctacaccggcggcggcagcacctactacgccgacagcgtgaagggcaggttcaccatcagcagggacaacagcaagaacaccctgtacctgcagatgaacagcctgagggccgaggacaccgccgtgtactactgcgccgccgacccctggagcgtgtacggcggcagctgcggcgtgaaggaccccaaccccaaggccttcaactactggggccagggcaccctggtgaccgtgagcagcggcggcggcggcagcggcggcggcggcagcggcggcggcggcagcggcggcggcggcagcgaggtgcagctgcaggagagcggcggcggcctggtgcagcccggcggcagcctgaggctgagctgcgccgccagcggctacccctacagcggcgactactgcatgggctggttcaggcaggcccccggcaaggagagggagggcgtggccgccttctacaccggcggcggcagcacctactacgccgacagcgtgaagggcaggttcaccatcagcagggacaacagcaagaacaccctgtacctgcagatgaacagcctgagggccgaggacaccgccgtgtactactgcgccgccgacccctggagcgtgtacggcggcagctgcggcgtgaaggaccccaaccccaaggccttcaactactggggccagggcaccctggtgaccgtgagcagcgagcccaagagctgcgacaagacccacacctgccccccctgccccgcccccgagctgctgggcggccccagcgtgttcctgttcccccccaagcccaaggacaccctgatgatcagcaggacccccgaggtgacctgcgtggtggtggacgtgagccacgaggaccccgaggtgaagttcaactggtacgtggacggcgtggaggtgcacaacgccaagaccaagcccagggaggagcagtacaacagcacctacagggtggtgagcgtgctgaccgtgctgcaccaggactggctgaacggcaaggagtacaagtgcaaggtgagcaacaaggccctgcccgcccccatcgagaagaccatcagcaaggccaagggccagcccagggagccccaggtgtacaccctgccccccagcagggaggagatgaccaagaaccaggtgagcctgacctgcctggtgaagggcttctaccccagcgacatcgccgtggagtgggagagcaacggccagcccgagaacaactacaagaccaccccccccgtgctggacagcgacggcagcttcttcctgtacagcaagctgaccgtggacaagagcaggtggcagcagggcaacgtgttcagctgcagcgtgatgcacgaggccctgcacaaccactacacccagaagagcctgagcctgagccccggcaag

SEQ ID NO: 55 - protein, 506 aa, Artificial Sequence
  HuNb21-HuNb66-Fc amino acid sequence
EVQLQESGGGLVQPGGSLRLSCAASGYPYSGDYCMGWFRQAPGKEREGVAAFYTGGGSTYYADSVKGRFTISRDNSKNTLYLQMNSLRAEDTAVYYCAADPWSVYGGSCGVKDPNPKAFNYWGQGTLVTVSSGGGGSGGGGSGGGGSGGGGSEVQLQESGGGLVQPGGSLRLSCAASGYTVSSNMGWFRQAPGKEREGVAAIYPDGATYYADSVKGRFTISRDNSENTLYLQMNSLRAEDTAMYYCAADLAFNGLGTLALHGYWGQGTLVTVSSEPKSCDKTHTCPPCPAPELLGGPSVFLFPPKPKDTLMISRTPEVTCVVVDVSHEDPEVKFNWYVDGVEVHNAKTKPREEQYNSTYRVVSVLTVLHQDWLNGKEYKCKVSNKALPAPIEKTISKAKGQPREPQVYTLPPSREEMTKNQVSLTCLVKGFYPSDIAVEWESNGQPENNYKTTPPVLDSDGSFFLYSKLTVDKSRWQQGNVFSCSVMHEALHNHYTQKSLSLSPGK

SEQ ID NO: 56 - DNA, 1518 bp, Artificial Sequence
  HuNb21-HuNb66-Fc nucleotide sequence
gaggtgcagctgcaggagagcggcggcggcctggtgcagcccggcggcagcctgaggctgagctgcgccgccagcggctacccctacagcggcgactactgcatgggctggttcaggcaggcccccggcaaggagagggagggcgtggccgccttctacaccggcggcggcagcacctactacgccgacagcgtgaagggcaggttcaccatcagcagggacaacagcaagaacaccctgtacctgcagatgaacagcctgagggccgaggacaccgccgtgtactactgcgccgccgacccctggagcgtgtacggcggcagctgcggcgtgaaggaccccaaccccaaggccttcaactactggggccagggcaccctggtgaccgtgagcagcggcggcggcggcagcggcggcggcggcagcggcggcggcggcagcggcggcggcggcagcgaggtgcagctgcaggagagcggcggcggcctggtgcagcccggcggcagcctgaggctgagctgcgccgccagcggctacaccgtgagcagcaacatgggctggttcaggcaggcccccggcaaggagagggagggcgtggccgccatctaccccgacggcgccacctactacgccgacagcgtgaagggcaggttcaccatcagcagggacaacagcgagaacaccctgtacctgcagatgaacagcctgagggccgaggacaccgccatgtactactgcgccgccgacctggccttcaacggcctgggcaccctggccctgcacggctactggggccagggcaccctggtgaccgtgagcagcgagcccaagagctgcgacaagacccacacctgccccccctgccccgcccccgagctgctgggcggccccagcgtgttcctgttcccccccaagcccaaggacaccctgatgatcagcaggacccccgaggtgacctgcgtggtggtggacgtgagccacgaggaccccgaggtgaagttcaactggtacgtggacggcgtggaggtgcacaacgccaagaccaagcccagggaggagcagtacaacagcacctacagggtggtgagcgtgctgaccgtgctgcaccaggactggctgaacggcaaggagtacaagtgcaaggtgagcaacaaggccctgcccgcccccatcgagaagaccatcagcaaggccaagggccagcccagggagccccaggtgtacaccctgccccccagcagggaggagatgaccaagaaccaggtgagcctgacctgcctggtgaagggcttctaccccagcgacatcgccgtggagtgggagagcaacggccagcccgagaacaactacaagaccaccccccccgtgctggacagcgacggcagcttcttcctgtacagcaagctgaccgtggacaagagcaggtggcagcagggcaacgtgttcagctgcagcgtgatgcacgaggccctgcacaaccactacacccagaagagcctgagcctgagccccggcaag

SEQ ID NO: 57 - protein, 496 aa, Artificial Sequence
  HuNb66-HuNb66-Fc amino acid sequence
EVQLQESGGGLVQPGGSLRLSCAASGYTVSSNMGWFRQAPGKEREGVAAIYPDGATYYADSVKGRFTISRDNSENTLYLQMNSLRAEDTAMYYCAADLAFNGLGTLALHGYWGQGTLVTVSSGGGGSGGGGSGGGGSGGGGSEVQLQESGGGLVQPGGSLRLSCAASGYTVSSNMGWFRQAPGKEREGVAAIYPDGATYYADSVKGRFTISRDNSENTLYLQMNSLRAEDTAMYYCAADLAFNGLGTLALHGYWGQGTLVTVSSEPKSCDKTHTCPPCPAPELLGGPSVFLFPPKPKDTLMISRTPEVTCVVVDVSHEDPEVKFNWYVDGVEVHNAKTKPREEQYNSTYRVVSVLTVLHQDWLNGKEYKCKVSNKALPAPIEKTISKAKGQPREPQVYTLPPSREEMTKNQVSLTCLVKGFYPSDIAVEWESNGQPENNYKTTPPVLDSDGSFFLYSKLTVDKSRWQQGNVFSCSVMHEALHNHYTQKSLSLSPGK

SEQ ID NO: 58 - DNA, 1488 bp, Artificial Sequence
  HuNb66-HuNb66-Fc nucleotide sequence
gaggtgcagctgcaggagagcggcggcggcctggtgcagcccggcggcagcctgaggctgagctgcgccgccagcggctacaccgtgagcagcaacatgggctggttcaggcaggcccccggcaaggagagggagggcgtggccgccatctaccccgacggcgccacctactacgccgacagcgtgaagggcaggttcaccatcagcagggacaacagcgagaacaccctgtacctgcagatgaacagcctgagggccgaggacaccgccatgtactactgcgccgccgacctggccttcaacggcctgggcaccctggccctgcacggctactggggccagggcaccctggtgaccgtgagcagcggcggcggcggcagcggcggcggcggcagcggcggcggcggcagcggcggcggcggcagcgaggtgcagctgcaggagagcggcggcggcctggtgcagcccggcggcagcctgaggctgagctgcgccgccagcggctacaccgtgagcagcaacatgggctggttcaggcaggcccccggcaaggagagggagggcgtggccgccatctaccccgacggcgccacctactacgccgacagcgtgaagggcaggttcaccatcagcagggacaacagcgagaacaccctgtacctgcagatgaacagcctgagggccgaggacaccgccatgtactactgcgccgccgacctggccttcaacggcctgggcaccctggccctgcacggctactggggccagggcaccctggtgaccgtgagcagcgagcccaagagctgcgacaagacccacacctgccccccctgccccgcccccgagctgctgggcggccccagcgtgttcctgttcccccccaagcccaaggacaccctgatgatcagcaggacccccgaggtgacctgcgtggtggtggacgtgagccacgaggaccccgaggtgaagttcaactggtacgtggacggcgtggaggtgcacaacgccaagaccaagcccagggaggagcagtacaacagcacctacagggtggtgagcgtgctgaccgtgctgcaccaggactggctgaacggcaaggagtacaagtgcaaggtgagcaacaaggccctgcccgcccccatcgagaagaccatcagcaaggccaagggccagcccagggagccccaggtgtacaccctgccccccagcagggaggagatgaccaagaaccaggtgagcctgacctgcctggtgaagggcttctaccccagcgacatcgccgtggagtgggagagcaacggccagcccgagaacaactacaagaccaccccccccgtgctggacagcgacggcagcttcttcctgtacagcaagctgaccgtggacaagagcaggtggcagcagggcaacgtgttcagctgcagcgtgatgcacgaggccctgcacaaccactacacccagaagagcctgagcctgagccccggcaag

SEQ ID NO: 59 - protein, 506 aa, Artificial Sequence
  HuNb66-HuNb21-Fc amino acid sequence
EVQLQESGGGLVQPGGSLRLSCAASGYTVSSNMGWFRQAPGKEREGVAAIYPDGATYYADSVKGRFTISRDNSENTLYLQMNSLRAEDTAMYYCAADLAFNGLGTLALHGYWGQGTLVTVSSGGGGSGGGGSGGGGSGGGGSEVQLQESGGGLVQPGGSLRLSCAASGYPYSGDYCMGWFRQAPGKEREGVAAFYTGGGSTYYADSVKGRFTISRDNSKNTLYLQMNSLRAEDTAVYYCAADPWSVYGGSCGVKDPNPKAFNYWGQGTLVTVSSEPKSCDKTHTCPPCPAPELLGGPSVFLFPPKPKDTLMISRTPEVTCVVVDVSHEDPEVKFNWYVDGVEVHNAKTKPREEQYNSTYRVVSVLTVLHQDWLNGKEYKCKVSNKALPAPIEKTISKAKGQPREPQVYTLPPSREEMTKNQVSLTCLVKGFYPSDIAVEWESNGQPENNYKTTPPVLDSDGSFFLYSKLTVDKSRWQQGNVFSCSVMHEALHNHYTQKSLSLSPGK

SEQ ID NO: 60 - DNA, 1518 bp, Artificial Sequence
  HuNb66-HuNb21-Fc nucleotide sequence
gaggtgcagctgcaggagagcggcggcggcctggtgcagcccggcggcagcctgaggctgagctgcgccgccagcggctacaccgtgagcagcaacatgggctggttcaggcaggcccccggcaaggagagggagggcgtggccgccatctaccccgacggcgccacctactacgccgacagcgtgaagggcaggttcaccatcagcagggacaacagcgagaacaccctgtacctgcagatgaacagcctgagggccgaggacaccgccatgtactactgcgccgccgacctggccttcaacggcctgggcaccctggccctgcacggctactggggccagggcaccctggtgaccgtgagcagcggcggcggcggcagcggcggcggcggcagcggcggcggcggcagcggcggcggcggcagcgaggtgcagctgcaggagagcggcggcggcctggtgcagcccggcggcagcctgaggctgagctgcgccgccagcggctacccctacagcggcgactactgcatgggctggttcaggcaggcccccggcaaggagagggagggcgtggccgccttctacaccggcggcggcagcacctactacgccgacagcgtgaagggcaggttcaccatcagcagggacaacagcaagaacaccctgtacctgcagatgaacagcctgagggccgaggacaccgccgtgtactactgcgccgccgacccctggagcgtgtacggcggcagctgcggcgtgaaggaccccaaccccaaggccttcaactactggggccagggcaccctggtgaccgtgagcagcgagcccaagagctgcgacaagacccacacctgccccccctgccccgcccccgagctgctgggcggccccagcgtgttcctgttcccccccaagcccaaggacaccctgatgatcagcaggacccccgaggtgacctgcgtggtggtggacgtgagccacgaggaccccgaggtgaagttcaactggtacgtggacggcgtggaggtgcacaacgccaagaccaagcccagggaggagcagtacaacagcacctacagggtggtgagcgtgctgaccgtgctgcaccaggactggctgaacggcaaggagtacaagtgcaaggtgagcaacaaggccctgcccgcccccatcgagaagaccatcagcaaggccaagggccagcccagggagccccaggtgtacaccctgccccccagcagggaggagatgaccaagaaccaggtgagcctgacctgcctggtgaagggcttctaccccagcgacatcgccgtggagtgggagagcaacggccagcccgagaacaactacaagaccaccccccccgtgctggacagcgacggcagcttcttcctgtacagcaagctgaccgtggacaagagcaggtggcagcagggcaacgtgttcagctgcagcgtgatgcacgaggccctgcacaaccactacacccagaagagcctgagcctgagccccggcaag

SEQ ID NO: 61 - protein, 274 aa, Artificial Sequence
  Amino acid sequence of divalent double epitope nanoantibody
EVQLQESGGGLVQPGGSLRLSCAASGYTVSSNMGWFRQAPGKEREGVAAIYPDGATYYADSVKGRFTISRDNSENTLYLQMNSLRAEDTAMYYCAADLAFNGLGTLALHGYWGQGTLVTVSSGGGGSGGGGSGGGGSGGGGSEVQLQESGGGLVQPGGSLRLSCAASGYPYSGDYCMGWFRQAPGKEREGVAAFYTGGGSTYYADSVKGRFTISRDNSKNTLYLQMNSLRAEDTAVYYCAADPWSVYGGSCGVKDPNPKAFNYWGQGTLVTVSS

SEQ ID NO: 62 - DNA, 822 bp, Artificial Sequence
  Nucleotide sequence of divalent double epitope nanoantibody
gaagttcaattgcaagaatctggtggtggtttggttcaaccaggtggttctttgagattgtcttgtgctgcttccggttacactgtttcttctaacatgggttggttcagacaagctccaggaaaggaaagagaaggtgttgctgctatctacccagatggtgctacttactacgctgattctgttaagggtagattcactatctctcgtgataactctgaaaacactttgtacttgcaaatgaactctttgagagctgaagatactgctatgtactactgtgctgctgatttggcttttaacggtttgggtaccttagctttgcatggttactggggtcaaggtactttggttactgtttcctctggtggtggtggttctggtggtggaggttctggtggaggtggttctggtggtggaggttctgaagttcaattgcaagaatctggaggtggtttggttcaacctggtggttctttgagattgtcttgtgctgcttctggttacccatattcaggagattactgtatgggttggtttagacaagctcctggaaaggaaagagaaggtgttgctgctttctatactggtggtggatctacttactacgctgattctgttaagggtagattcactatttccagagataactctaagaacactttgtacttgcaaatgaactctttgagagctgaagatactgctgtttactactgtgctgctgatccatggtctgtttacggtggttcttgtggtgttaaggatccaaacccaaaggctttcaactactggggtcaaggtactttggttactgtttcttcc

SEQ ID NO: 63 - protein, 232 aa, Artificial Sequence
  Fc fragment
EPKSCDKTHTCPPCPAPELLGGPSVFLFPPKPKDTLMISRTPEVTCVVVDVSHEDPEVKFNWYVDGVEVHNAKTKPREEQYNSTYRVVSVLTVLHQDWLNGKEYKCKVSNKALPAPIEKTISKAKGQPREPQVYTLPPSREEMTKNQVSLTCLVKGFYPSDIAVEWESNGQPENNYKTTPPVLDSDGSFFLYSKLTVDKSRWQQGNVFSCSVMHEALHNHYTQKSLSLSPGK